European Patent Application EP 4 648 053 A2, published November 12, 2025. Title: DISTINGUISHING METHYLATION LEVELS IN COMPLEX BIOLOGICAL SAMPLES. Applicant: Illumina, Inc. Application EP. The sequence listing filed with the application follows.

SEQUENCE LISTING (9 sequences)

SEQ ID NO: 1 - DNA, 22 bp, synthetic construct
  misc_feature 1..22: note = Probe
  modified_base 12: mod_base = OTHER; note = Methylated
  modified_base 16: mod_base = OTHER; note = Methylated
  source 1..22: mol_type = other DNA
acgatcgccttcgaccgtcgaa

SEQ ID NO: 2 - DNA, 22 bp, synthetic construct
  misc_feature 1..22: note = Probe
  misc_feature 2: note = uracil that is expected to result from bisulfate conversion
  misc_feature 6: note = uracil that is expected to result from bisulfate conversion
  misc_feature 8..9: note = uracil that is expected to result from bisulfate conversion
  modified_base 12: mod_base = OTHER; note = Methylated
  misc_feature 15: note = uracil that is expected to result from bisulfate conversion
  modified_base 16: mod_base = OTHER; note = Methylated
  misc_feature 19: note = uracil that is expected to result from bisulfate conversion
  source 1..22: mol_type = other DNA
angatngnnttcgancgtngaa

SEQ ID NO: 3 - DNA, 22 bp, synthetic construct
  misc_feature 1..22: note = Probe
  source 1..22: mol_type = other DNA
atgattgttttcgatcgttgaa

SEQ ID NO: 4 - DNA, 22 bp, synthetic construct
  misc_feature 1..22: note = Probe
  modified_base 16: mod_base = OTHER; note = Methylated
  source 1..22: mol_type = other DNA
atgatagccttcgaccgtagaa

SEQ ID NO: 5 - DNA, 22 bp, synthetic construct
  misc_feature 1..22: note = Probe
  misc_feature 8..9: note = uracil that is expected to result from bisulfate conversion
  misc_feature 12: note = uracil that is expected to result from bisulfate conversion
  modified_base 16: mod_base = OTHER; note = Methylated
  source 1..22: mol_type = other DNA
atgatagnnttngaccgtagaa

SEQ ID NO: 6 - DNA, 22 bp, synthetic construct
  misc_feature 1..22: note = Probe
  source 1..22: mol_type = other DNA
atgatagtttttgaccgtagaa

SEQ ID NO: 7 - DNA, 22 bp, synthetic construct
  misc_feature 1..22: note = Probe
  source 1..22: mol_type = other DNA
ttcgacgatcgaaaacgatcgt

SEQ ID NO: 8 - DNA, 22 bp, synthetic construct
  misc_feature 1..22: note = Probe
  source 1..22: mol_type = other DNA
ttcaacaatcaaaaacaatcat

SEQ ID NO: 9 - DNA, 22 bp, synthetic construct
  misc_feature 1..22: note = Probe
  source 1..22: mol_type = other DNA
ttctacrgtcraaaactatcat